European Patent Application EP 4 141 028 A1, published March 1, 2023. Title: Personalized vNAR-based chimeric antigen receptors (vNAR-CAR) for the treatment of clonal B-and T cell malignancies, and methods for producing vNAR-CARs. Applicant: Johann Wolfgang Goethe-Universität Frankfurt am Main Technische Universität Darmstadt. The sequence listing filed with the application follows.

SEQUENCE LISTING (5 sequences)

SEQ ID NO: 1 - protein, 348 aa, artificial sequence
  vNAR-CAR sequence
MDWIWRILFLVGAATGAHSEQKLISEEDLMAARLEQTPTTTTKEAGESLTINCVLKGSKYALGNTYWYFTKKGATKKASLSTGGRYSDTKNTASKSFSLRISDLRVEDSGTYHCEAYFAGFHYMLKRHIEGGGTTLTVKGGGGSGGGGSGGGGSGGGGSLQTRGLDKPFWVLVVVGGVLACYSLLVTVAFIIFWVRSKRSRLLHSDYMNMTPRRPGPTRKHYQPYAPPRDFAAYRSRVKFSRSADAPAYQQGQNQLYNELNLGRREEYDVLDKRRGRDPEMGGKPRRKNPQEGLYNELQKDKMAEAYSEIGMKGERRRGKGHDGLYQGLSTATKDTYDALHMQALPPR

SEQ ID NO: 2 - DNA, 1047 bp, artificial sequence
  vNAR-CAR sequence
atggactggatttggagaatcctgttcctcgtgggagccgccacaggcgctcattctgagcagaagctgatctccgaagaggacctgatggctgctagactggaacagacccctaccaccaccacaaaagaggccggcgagagcctgaccatcaactgtgtgctgaagggctctaagtacgccctgggcaacacctactggtacttcaccaagaagggcgccacaaagaaggccagcctgtctacaggcggcagatacagcgacaccaagaacaccgccagcaagagcttcagcctgcggatcagcgatctgagagtggaagatagcggcacctaccactgcgaggcctactttgccggcttccactacatgctgaagcggcacattgaaggcggcggaaccacactgaccgtgaaaggcggaggcggaagtggaggcggaggaagcggagggggaggatcaggcggcggagggtccctgcagaccaggggcctggacaagcccttctgggtgctggtcgtggtcggcggcgtgctggcctgttacagcctgctggtcaccgtggccttcatcatcttttgggtccgcagcaagagaagccggctgctgcactccgactacatgaacatgacccccagacggcctggccccaccagaaagcactaccagccctacgcccctcctagagatttcgccgcctaccggtccagagtgaagttcagcagatccgccgacgcccctgcctatcagcagggccagaaccagctgtacaacgagctgaacctgggcagacgggaggaatacgacgtgctggacaagagaagaggccgggaccctgagatgggcggcaagcccagacggaagaacccccaggaaggcctgtataacgaactgcagaaagacaagatggccgaggcctacagcgagatcggcatgaagggcgagcggagaagaggcaagggccacgacggcctgtaccagggcctgagcaccgccaccaaggacacctacgacgccctgcacatgcaggctctgccacctagataa

SEQ ID NO: 3 - protein, 110 aa, artificial sequence
  vNAR sequence
MAARLEQTPTTTTKEAGESLTINCVLKGSKYALGNTYWYFTKKGATKKASLSTGGRYSDTKNTASKSFSLRISDLRVEDSGTYHCEAYFAGFHYMLKRHIEGGGTTLTVK

SEQ ID NO: 4 - DNA, 330 bp, artificial sequence
  vNAR sequence
atggctgctagactggaacagacccctaccaccaccacaaaagaggccggcgagagcctgaccatcaactgtgtgctgaagggctctaagtacgccctgggcaacacctactggtacttcaccaagaagggcgccacaaagaaggccagcctgtctacaggcggcagatacagcgacaccaagaacaccgccagcaagagcttcagcctgcggatcagcgatctgagagtggaagatagcggcacctaccactgcgaggcctactttgccggcttccactacatgctgaagcggcacattgaaggcggcggaaccacactgaccgtgaaa

SEQ ID NO: 5 - protein, 5 aa, artificial sequence
  linker sequence
GGGGS